European Patent Application EP 4 317 177 A1, published February 7, 2024. Title: NOVEL CORONAVIRUS S-RBD TRIMERIC PROTEIN VACCINE, PREPARATION METHOD THEREFOR, AND APPLICATION THEREOF. Applicant: NATIONAL VACCINE AND SERUM INSTITUTE(NVSI). The sequence listing filed with the application follows.

SEQUENCE LISTING (4 sequences)

SEQ ID NO: 1 - protein, 658 aa, Virus
MRVQPTESIVRFPNITNLCPFGEVFNATRFASVYAWNRKRISNCVADYSVLYNSASFSTFKCYGVSPTKLNDLCFTNVYADSFVIRGDEVRQIAPGQTGKIADYNYKLPDDFTGCVIAWNSNNLDSKVGGNYNYLYRLFRKSNLKPFERDISTEIYQAGSTPCNGVEGFNCYFPLQSYGFQPTNGVGYQPYRVVVLSFELLHAPATVCGPKKSTNLVKNKRVQPTESIVRFPNITNLCPFGEVFNATRFASVYAWNRKRISNCVADYSVLYNSASFSTFKCYGVSPTKLNDLCFTNVYADSFVIRGDEVRQIAPGQTGKIADYNYKLPDDFTGCVIAWNSNNLDSKVGGNYNYLYRLFRKSNLKPFERDISTEIYQAGSTPCNGVEGFNCYFPLQSYGFQPTNGVGYQPYRVVVLSFELLHAPATVCGPKKSTNLVKNKRVQPTESIVRFPNITNLCPFGEVFNATRFASVYAWNRKRISNCVADYSVLYNSASFSTFKCYGVSPTKLNDLCFTNVYADSFVIRGDEVRQIAPGQTGKIADYNYKLPDDFTGCVIAWNSNNLDSKVGGNYNYLYRLFRKSNLKPFERDISTEIYQAGSTPCNGVEGFNCYFPLQSYGFQPTNGVGYQPYRVVVLSFELLHAPATVCGPKKSTNLVKNK

SEQ ID NO: 2 - DNA, 1977 bp, Artificial
atgagagtgcagcccacagagtcaattgtgagattccccaatatcactaacctgtgcccctttggggaggtgttcaatgccacaagatttgcttctgtgtatgcctggaatagaaagagaatcagtaactgtgttgctgactactctgtgctgtacaattctgcctctttcagcacattcaaatgttatggggttagccccaccaaactaaatgacctgtgcttcaccaatgtgtatgctgacagctttgtgatcagaggtgatgaagtgagacaaattgcccctgggcagactggcaagatagctgactacaattacaagctgcctgatgactttactggctgtgtgattgcctggaatagcaataacctggacagcaaggtggggggcaactataactacctatacagattgtttagaaagtccaatttgaaaccctttgagagagatatcagcactgagatctatcaagctggcagcaccccctgtaatggggtggaggggttcaactgctatttccccttacagagctatggctttcagcccaccaatggggtgggctatcagccctacagagtggtggtgctgtcttttgaactacttcatgcccctgccacagtgtgtggccccaaaaaaagcacaaacctggtgaaaaacaagagagtgcagccaacagagagcattgtgagattccctaacataaccaatctgtgtccctttggtgaggtttttaatgctactagatttgcctctgtgtatgcctggaacagaaaaagaatctcaaactgtgtggctgactattcagtcctctacaactcagctagctttagcaccttcaaatgctatggtgtcagtcccaccaaactgaatgacctttgtttcaccaatgtctatgctgacagctttgtgatcagaggggatgaagtgagacaaatagcccctgggcagactggcaagatagctgattacaactataaactgcctgatgatttcactggctgtgtcattgcctggaactcaaataatctagacagcaaggtaggtggcaattataactacctctataggctgtttaggaaaagtaacctgaaaccctttgagagagacattagcacagagatttatcaagctggctcaacaccctgtaatggtgtggagggctttaactgctacttccccctgcagagctatggctttcagccaaccaatggagtgggctatcagccctatagagtagttgtgctgagctttgagctgctgcatgcccctgccacagtgtgtggccctaagaaaagcaccaacttggtcaaaaataagagagtacaacccacagagtccattgtgagatttcccaacatcactaatttgtgtccttttggggaggtcttcaatgccacaagatttgcctctgtgtatgcctggaacagaaagagaatcagcaactgtgtggctgactactctgtgctgtacaactctgcctccttcagcaccttcaagtgctatggggtgagccccaccaagctcaatgacttatgcttcaccaatgtgtatgctgacagctttgtgattagaggggatgaggtcagacagattgcccctggccaaactggaaaaattgctgactacaactacaaactgcctgatgactttactggctgtgtgattgcctggaactccaacaaccttgatagcaaggttggggggaattataactatctgtacagactattcagaaagagcaacctgaaaccctttgagagagacatctcaacagaaatatatcaagctggctccactccatgcaatggggtggagggattcaattgttacttccccctgcagtcatatggctttcaacccaccaatggggtgggctaccaaccttacagagtggtagtactttcctttgagctacttcatgcccctgccacagtgtgtggccccaagaaaagcaccaatctggtaaagaataagtga

SEQ ID NO: 3 - protein, 439 aa, Virus
MRVQPTESIVRFPNITNLCPFGEVFNATRFASVYAWNRKRISNCVADYSVLYNSASFSTFKCYGVSPTKLNDLCFTNVYADSFVIRGDEVRQIAPGQTGKIADYNYKLPDDFTGCVIAWNSNNLDSKVGGNYNYLYRLFRKSNLKPFERDISTEIYQAGSTPCNGVEGFNCYFPLQSYGFQPTNGVGYQPYRVVVLSFELLHAPATVCGPKKSTNLVKNKRVQPTESIVRFPNITNLCPFGEVFNATRFASVYAWNRKRISNCVADYSVLYNSASFSTFKCYGVSPTKLNDLCFTNVYADSFVIRGDEVRQIAPGQTGKIADYNYKLPDDFTGCVIAWNSNNLDSKVGGNYNYLYRLFRKSNLKPFERDISTEIYQAGSTPCNGVEGFNCYFPLQSYGFQPTNGVGYQPYRVVVLSFELLHAPATVCGPKKSTNLVKNK

SEQ ID NO: 4 - DNA, 1320 bp, Artificial
atgagagtgcagcccacagagtcaattgtgagattccccaatatcactaacctgtgcccctttggggaggtgttcaatgccacaagatttgcttctgtgtatgcctggaatagaaagagaatcagtaactgtgttgctgactactctgtgctgtacaattctgcctctttcagcacattcaaatgttatggggttagccccaccaaactaaatgacctgtgcttcaccaatgtgtatgctgacagctttgtgatcagaggtgatgaagtgagacaaattgcccctgggcagactggcaagatagctgactacaattacaagctgcctgatgactttactggctgtgtgattgcctggaatagcaataacctggacagcaaggtggggggcaactataactacctatacagattgtttagaaagtccaatttgaaaccctttgagagagatatcagcactgagatctatcaagctggcagcaccccctgtaatggggtggaggggttcaactgctatttccccttacagagctatggctttcagcccaccaatggggtgggctatcagccctacagagtggtggtgctgtcttttgaactacttcatgcccctgccacagtgtgtggccccaaaaaaagcacaaacctggtgaaaaacaagagagtgcagccaacagagagcattgtgagattccctaacataaccaatctgtgtccctttggtgaggtttttaatgctactagatttgcctctgtgtatgcctggaacagaaaaagaatctcaaactgtgtggctgactattcagtcctctacaactcagctagctttagcaccttcaaatgctatggtgtcagtcccaccaaactgaatgacctttgtttcaccaatgtctatgctgacagctttgtgatcagaggggatgaagtgagacaaatagcccctgggcagactggcaagatagctgattacaactataaactgcctgatgatttcactggctgtgtcattgcctggaactcaaataatctagacagcaaggtaggtggcaattataactacctctataggctgtttaggaaaagtaacctgaaaccctttgagagagacattagcacagagatttatcaagctggctcaacaccctgtaatggtgtggagggctttaactgctacttccccctgcagagctatggctttcagccaaccaatggagtgggctatcagccctatagagtagttgtgctgagctttgagctgctgcatgcccctgccacagtgtgtggccctaagaaaagcaccaacttggtcaaaaataagtga